European Patent Application EP 4 800 103 A1, published September 2, 2026. Title: A novel phosphoribosyl aminimidazole-succinocarboxamide synthase variant and a method of producing purine nucleotides using the same. Applicant: CJ CheilJedang Corporation. Application KR. The sequence listing filed with the application follows.

SEQUENCE LISTING (37 sequences)

SEQ ID NO: 1 - DNA, 39 bp, synthetic construct
  source 1..39: mol_type = other DNA
ttcgagctcggtacccgtcagcagtggaacgaaggcgac

SEQ ID NO: 2 - DNA, 38 bp, synthetic construct
  source 1..38: mol_type = other DNA
ctctagaggatccccagatatcggtcaggtggtcatcg

SEQ ID NO: 3 - DNA, 18 bp, synthetic construct
  source 1..18: mol_type = other DNA
ggtaagagtccagaagaa

SEQ ID NO: 4 - DNA, 18 bp, synthetic construct
  source 1..18: mol_type = other DNA
cgcatccactcatattca

SEQ ID NO: 5 - protein, 295 aa, Corynebacterium stationis
MRPQLSDYQHVSSGKVRDIYEVDDNTLLMVVTDRISAYDFALEPAIPDKGRVLTATTMFFFDAIDFPNHLAGPIDDARIPEEVLGRAIIVKKLNMLPFECVARGYLTGSGLKEYNANGTVCGIELPEGLVEASRLPEPIFTPATKAEQGDHDENVSFERVVQDLGQERAEQLRDETLRIYSAAAKIAEEKGIILADTKFEFGLDSEGNLVLGDEVLTPDSSRYWPADTYAEGIVQPSFDKQYVRNWLTSEESGWDVESETQPPVLPDDIVAATRLRYIEAYERLSGKRFIDFIGG

SEQ ID NO: 6 - DNA, 37 bp, synthetic construct
  source 1..37: mol_type = other DNA
cgatgggtcctgccaaagcgttcgggaaatcgatggc

SEQ ID NO: 7 - DNA, 36 bp, synthetic construct
  source 1..36: mol_type = other DNA
tcgatttcccgaacgctttggcaggacccatcgatg

SEQ ID NO: 8 - DNA, 37 bp, synthetic construct
  source 1..37: mol_type = other DNA
cgatgggtcctgccaacacgttcgggaaatcgatggc

SEQ ID NO: 9 - DNA, 36 bp, synthetic construct
  source 1..36: mol_type = other DNA
tcgatttcccgaacgtgttggcaggacccatcgatg

SEQ ID NO: 10 - DNA, 37 bp, synthetic construct
  source 1..37: mol_type = other DNA
cgatgggtcctgccaagaggttcgggaaatcgatggc

SEQ ID NO: 11 - DNA, 36 bp, synthetic construct
  source 1..36: mol_type = other DNA
tcgatttcccgaacctcttggcaggacccatcgatg

SEQ ID NO: 12 - DNA, 37 bp, synthetic construct
  source 1..37: mol_type = other DNA
cgatgggtcctgccaaggtgttcgggaaatcgatggc

SEQ ID NO: 13 - DNA, 36 bp, synthetic construct
  source 1..36: mol_type = other DNA
tcgatttcccgaacaccttggcaggacccatcgatg

SEQ ID NO: 14 - DNA, 37 bp, synthetic construct
  source 1..37: mol_type = other DNA
cgatgggtcctgccaagttgttcgggaaatcgatggc

SEQ ID NO: 15 - DNA, 36 bp, synthetic construct
  source 1..36: mol_type = other DNA
tcgatttcccgaacaacttggcaggacccatcgatg

SEQ ID NO: 16 - DNA, 37 bp, synthetic construct
  source 1..37: mol_type = other DNA
cgatgggtcctgccaatgggttcgggaaatcgatggc

SEQ ID NO: 17 - DNA, 36 bp, synthetic construct
  source 1..36: mol_type = other DNA
tcgatttcccgaacccattggcaggacccatcgatg

SEQ ID NO: 18 - DNA, 37 bp, synthetic construct
  source 1..37: mol_type = other DNA
cgatgggtcctgccaacgagttcgggaaatcgatggc

SEQ ID NO: 19 - DNA, 36 bp, synthetic construct
  source 1..36: mol_type = other DNA
tcgatttcccgaactcgttggcaggacccatcgatg

SEQ ID NO: 20 - protein, 295 aa, synthetic construct
MRPQLSDYQHVSSGKVRDIYEVDDNTLLMVVTDRISAYDFALEPAIPDKGRVLTATTMFFFDAIDFPNQLAGPIDDARIPEEVLGRAIIVKKLNMLPFECVARGYLTGSGLKEYNANGTVCGIELPEGLVEASRLPEPIFTPATKAEQGDHDENVSFERVVQDLGQERAEQLRDETLRIYSAAAKIAEEKGIILADTKFEFGLDSEGNLVLGDEVLTPDSSRYWPADTYAEGIVQPSFDKQYVRNWLTSEESGWDVESETQPPVLPDDIVAATRLRYIEAYERLSGKRFIDFIGG

SEQ ID NO: 21 - protein, 295 aa, synthetic construct
MRPQLSDYQHVSSGKVRDIYEVDDNTLLMVVTDRISAYDFALEPAIPDKGRVLTATTMFFFDAIDFPNALAGPIDDARIPEEVLGRAIIVKKLNMLPFECVARGYLTGSGLKEYNANGTVCGIELPEGLVEASRLPEPIFTPATKAEQGDHDENVSFERVVQDLGQERAEQLRDETLRIYSAAAKIAEEKGIILADTKFEFGLDSEGNLVLGDEVLTPDSSRYWPADTYAEGIVQPSFDKQYVRNWLTSEESGWDVESETQPPVLPDDIVAATRLRYIEAYERLSGKRFIDFIGG

SEQ ID NO: 22 - protein, 295 aa, synthetic construct
MRPQLSDYQHVSSGKVRDIYEVDDNTLLMVVTDRISAYDFALEPAIPDKGRVLTATTMFFFDAIDFPNVLAGPIDDARIPEEVLGRAIIVKKLNMLPFECVARGYLTGSGLKEYNANGTVCGIELPEGLVEASRLPEPIFTPATKAEQGDHDENVSFERVVQDLGQERAEQLRDETLRIYSAAAKIAEEKGIILADTKFEFGLDSEGNLVLGDEVLTPDSSRYWPADTYAEGIVQPSFDKQYVRNWLTSEESGWDVESETQPPVLPDDIVAATRLRYIEAYERLSGKRFIDFIGG

SEQ ID NO: 23 - protein, 295 aa, synthetic construct
MRPQLSDYQHVSSGKVRDIYEVDDNTLLMVVTDRISAYDFALEPAIPDKGRVLTATTMFFFDAIDFPNLLAGPIDDARIPEEVLGRAIIVKKLNMLPFECVARGYLTGSGLKEYNANGTVCGIELPEGLVEASRLPEPIFTPATKAEQGDHDENVSFERVVQDLGQERAEQLRDETLRIYSAAAKIAEEKGIILADTKFEFGLDSEGNLVLGDEVLTPDSSRYWPADTYAEGIVQPSFDKQYVRNWLTSEESGWDVESETQPPVLPDDIVAATRLRYIEAYERLSGKRFIDFIGG

SEQ ID NO: 24 - protein, 295 aa, synthetic construct
MRPQLSDYQHVSSGKVRDIYEVDDNTLLMVVTDRISAYDFALEPAIPDKGRVLTATTMFFFDAIDFPNTLAGPIDDARIPEEVLGRAIIVKKLNMLPFECVARGYLTGSGLKEYNANGTVCGIELPEGLVEASRLPEPIFTPATKAEQGDHDENVSFERVVQDLGQERAEQLRDETLRIYSAAAKIAEEKGIILADTKFEFGLDSEGNLVLGDEVLTPDSSRYWPADTYAEGIVQPSFDKQYVRNWLTSEESGWDVESETQPPVLPDDIVAATRLRYIEAYERLSGKRFIDFIGG

SEQ ID NO: 25 - protein, 295 aa, synthetic construct
MRPQLSDYQHVSSGKVRDIYEVDDNTLLMVVTDRISAYDFALEPAIPDKGRVLTATTMFFFDAIDFPNNLAGPIDDARIPEEVLGRAIIVKKLNMLPFECVARGYLTGSGLKEYNANGTVCGIELPEGLVEASRLPEPIFTPATKAEQGDHDENVSFERVVQDLGQERAEQLRDETLRIYSAAAKIAEEKGIILADTKFEFGLDSEGNLVLGDEVLTPDSSRYWPADTYAEGIVQPSFDKQYVRNWLTSEESGWDVESETQPPVLPDDIVAATRLRYIEAYERLSGKRFIDFIGG

SEQ ID NO: 26 - protein, 295 aa, synthetic construct
MRPQLSDYQHVSSGKVRDIYEVDDNTLLMVVTDRISAYDFALEPAIPDKGRVLTATTMFFFDAIDFPNPLAGPIDDARIPEEVLGRAIIVKKLNMLPFECVARGYLTGSGLKEYNANGTVCGIELPEGLVEASRLPEPIFTPATKAEQGDHDENVSFERVVQDLGQERAEQLRDETLRIYSAAAKIAEEKGIILADTKFEFGLDSEGNLVLGDEVLTPDSSRYWPADTYAEGIVQPSFDKQYVRNWLTSEESGWDVESETQPPVLPDDIVAATRLRYIEAYERLSGKRFIDFIGG

SEQ ID NO: 27 - protein, 295 aa, synthetic construct
MRPQLSDYQHVSSGKVRDIYEVDDNTLLMVVTDRISAYDFALEPAIPDKGRVLTATTMFFFDAIDFPNSLAGPIDDARIPEEVLGRAIIVKKLNMLPFECVARGYLTGSGLKEYNANGTVCGIELPEGLVEASRLPEPIFTPATKAEQGDHDENVSFERVVQDLGQERAEQLRDETLRIYSAAAKIAEEKGIILADTKFEFGLDSEGNLVLGDEVLTPDSSRYWPADTYAEGIVQPSFDKQYVRNWLTSEESGWDVESETQPPVLPDDIVAATRLRYIEAYERLSGKRFIDFIGG

SEQ ID NO: 28 - DNA, 888 bp, Corynebacterium stationis
  source 1..888: mol_type = other DNA
atgcgcccacagctttctgattatcagcacgtatcctccggcaaagtccgcgatatctacgaagtagatgacaacactttgctcatggtggtcaccgaccgcatctccgcctatgacttcgcactagagccagccatccccgataaaggccgggttcttaccgcaaccaccatgttcttcttcgacgccatcgatttcccgaaccatttggcaggacccatcgatgatgcgcggattccagaagaagtattgggccgagcgatcatcgttaagaagctcaacatgctgccctttgagtgcgttgcccgcggttacctcaccggttccggcttgaaggaatacaacgctaacggcaccgtgtgcggcatcgagctgccagaaggcttggttgaggcgtcgcgtctgccagagccaattttcaccccagccaccaaggcagagcagggcgaccacgatgaaaacgtcagcttcgagcgcgtggtgcaggaccttggccaagagcgcgcagagcagcttcgcgatgaaaccctgcgcatctactccgccgccgccaagattgccgaagaaaagggcatcatcttggctgatacgaagtttgaattcggccttgattccgaaggcaatctggtcttgggcgatgaagtacttacgcctgattcctcccggtactggccagcagacacctacgcggaaggcattgtgcagcccagctttgacaagcagtacgtgcgcaactggttgacctcggaggaatccggctgggatgtggagtcggaaacccagccgccagtgcttcccgatgacatcgtcgccgccacccgcctgcgctacatcgaggcttatgagcgcttgtccggcaagcgtttcatcgacttcattggcggttaa

SEQ ID NO: 29 - DNA, 888 bp, synthetic construct
  source 1..888: mol_type = other DNA
atgcgcccacagctttctgattatcagcacgtatcctccggcaaagtccgcgatatctacgaagtagatgacaacactttgctcatggtggtcaccgaccgcatctccgcctatgacttcgcactagagccagccatccccgataaaggccgggttcttaccgcaaccaccatgttcttcttcgacgccatcgatttcccgaaccagttggcaggacccatcgatgatgcgcggattccagaagaagtattgggccgagcgatcatcgttaagaagctcaacatgctgccctttgagtgcgttgcccgcggttacctcaccggttccggcttgaaggaatacaacgctaacggcaccgtgtgcggcatcgagctgccagaaggcttggttgaggcgtcgcgtctgccagagccaattttcaccccagccaccaaggcagagcagggcgaccacgatgaaaacgtcagcttcgagcgcgtggtgcaggaccttggccaagagcgcgcagagcagcttcgcgatgaaaccctgcgcatctactccgccgccgccaagattgccgaagaaaagggcatcatcttggctgatacgaagtttgaattcggccttgattccgaaggcaatctggtcttgggcgatgaagtacttacgcctgattcctcccggtactggccagcagacacctacgcggaaggcattgtgcagcccagctttgacaagcagtacgtgcgcaactggttgacctcggaggaatccggctgggatgtggagtcggaaacccagccgccagtgcttcccgatgacatcgtcgccgccacccgcctgcgctacatcgaggcttatgagcgcttgtccggcaagcgtttcatcgacttcattggcggttaa

SEQ ID NO: 30 - DNA, 888 bp, synthetic construct
  source 1..888: mol_type = other DNA
atgcgcccacagctttctgattatcagcacgtatcctccggcaaagtccgcgatatctacgaagtagatgacaacactttgctcatggtggtcaccgaccgcatctccgcctatgacttcgcactagagccagccatccccgataaaggccgggttcttaccgcaaccaccatgttcttcttcgacgccatcgatttcccgaacgctttggcaggacccatcgatgatgcgcggattccagaagaagtattgggccgagcgatcatcgttaagaagctcaacatgctgccctttgagtgcgttgcccgcggttacctcaccggttccggcttgaaggaatacaacgctaacggcaccgtgtgcggcatcgagctgccagaaggcttggttgaggcgtcgcgtctgccagagccaattttcaccccagccaccaaggcagagcagggcgaccacgatgaaaacgtcagcttcgagcgcgtggtgcaggaccttggccaagagcgcgcagagcagcttcgcgatgaaaccctgcgcatctactccgccgccgccaagattgccgaagaaaagggcatcatcttggctgatacgaagtttgaattcggccttgattccgaaggcaatctggtcttgggcgatgaagtacttacgcctgattcctcccggtactggccagcagacacctacgcggaaggcattgtgcagcccagctttgacaagcagtacgtgcgcaactggttgacctcggaggaatccggctgggatgtggagtcggaaacccagccgccagtgcttcccgatgacatcgtcgccgccacccgcctgcgctacatcgaggcttatgagcgcttgtccggcaagcgtttcatcgacttcattggcggttaa

SEQ ID NO: 31 - DNA, 888 bp, synthetic construct
  source 1..888: mol_type = other DNA
atgcgcccacagctttctgattatcagcacgtatcctccggcaaagtccgcgatatctacgaagtagatgacaacactttgctcatggtggtcaccgaccgcatctccgcctatgacttcgcactagagccagccatccccgataaaggccgggttcttaccgcaaccaccatgttcttcttcgacgccatcgatttcccgaacgtgttggcaggacccatcgatgatgcgcggattccagaagaagtattgggccgagcgatcatcgttaagaagctcaacatgctgccctttgagtgcgttgcccgcggttacctcaccggttccggcttgaaggaatacaacgctaacggcaccgtgtgcggcatcgagctgccagaaggcttggttgaggcgtcgcgtctgccagagccaattttcaccccagccaccaaggcagagcagggcgaccacgatgaaaacgtcagcttcgagcgcgtggtgcaggaccttggccaagagcgcgcagagcagcttcgcgatgaaaccctgcgcatctactccgccgccgccaagattgccgaagaaaagggcatcatcttggctgatacgaagtttgaattcggccttgattccgaaggcaatctggtcttgggcgatgaagtacttacgcctgattcctcccggtactggccagcagacacctacgcggaaggcattgtgcagcccagctttgacaagcagtacgtgcgcaactggttgacctcggaggaatccggctgggatgtggagtcggaaacccagccgccagtgcttcccgatgacatcgtcgccgccacccgcctgcgctacatcgaggcttatgagcgcttgtccggcaagcgtttcatcgacttcattggcggttaa

SEQ ID NO: 32 - DNA, 888 bp, synthetic construct
  source 1..888: mol_type = other DNA
atgcgcccacagctttctgattatcagcacgtatcctccggcaaagtccgcgatatctacgaagtagatgacaacactttgctcatggtggtcaccgaccgcatctccgcctatgacttcgcactagagccagccatccccgataaaggccgggttcttaccgcaaccaccatgttcttcttcgacgccatcgatttcccgaacctcttggcaggacccatcgatgatgcgcggattccagaagaagtattgggccgagcgatcatcgttaagaagctcaacatgctgccctttgagtgcgttgcccgcggttacctcaccggttccggcttgaaggaatacaacgctaacggcaccgtgtgcggcatcgagctgccagaaggcttggttgaggcgtcgcgtctgccagagccaattttcaccccagccaccaaggcagagcagggcgaccacgatgaaaacgtcagcttcgagcgcgtggtgcaggaccttggccaagagcgcgcagagcagcttcgcgatgaaaccctgcgcatctactccgccgccgccaagattgccgaagaaaagggcatcatcttggctgatacgaagtttgaattcggccttgattccgaaggcaatctggtcttgggcgatgaagtacttacgcctgattcctcccggtactggccagcagacacctacgcggaaggcattgtgcagcccagctttgacaagcagtacgtgcgcaactggttgacctcggaggaatccggctgggatgtggagtcggaaacccagccgccagtgcttcccgatgacatcgtcgccgccacccgcctgcgctacatcgaggcttatgagcgcttgtccggcaagcgtttcatcgacttcattggcggttaa

SEQ ID NO: 33 - DNA, 888 bp, synthetic construct
  source 1..888: mol_type = other DNA
atgcgcccacagctttctgattatcagcacgtatcctccggcaaagtccgcgatatctacgaagtagatgacaacactttgctcatggtggtcaccgaccgcatctccgcctatgacttcgcactagagccagccatccccgataaaggccgggttcttaccgcaaccaccatgttcttcttcgacgccatcgatttcccgaacaccttggcaggacccatcgatgatgcgcggattccagaagaagtattgggccgagcgatcatcgttaagaagctcaacatgctgccctttgagtgcgttgcccgcggttacctcaccggttccggcttgaaggaatacaacgctaacggcaccgtgtgcggcatcgagctgccagaaggcttggttgaggcgtcgcgtctgccagagccaattttcaccccagccaccaaggcagagcagggcgaccacgatgaaaacgtcagcttcgagcgcgtggtgcaggaccttggccaagagcgcgcagagcagcttcgcgatgaaaccctgcgcatctactccgccgccgccaagattgccgaagaaaagggcatcatcttggctgatacgaagtttgaattcggccttgattccgaaggcaatctggtcttgggcgatgaagtacttacgcctgattcctcccggtactggccagcagacacctacgcggaaggcattgtgcagcccagctttgacaagcagtacgtgcgcaactggttgacctcggaggaatccggctgggatgtggagtcggaaacccagccgccagtgcttcccgatgacatcgtcgccgccacccgcctgcgctacatcgaggcttatgagcgcttgtccggcaagcgtttcatcgacttcattggcggttaa

SEQ ID NO: 34 - DNA, 888 bp, synthetic construct
  source 1..888: mol_type = other DNA
atgcgcccacagctttctgattatcagcacgtatcctccggcaaagtccgcgatatctacgaagtagatgacaacactttgctcatggtggtcaccgaccgcatctccgcctatgacttcgcactagagccagccatccccgataaaggccgggttcttaccgcaaccaccatgttcttcttcgacgccatcgatttcccgaacaacttggcaggacccatcgatgatgcgcggattccagaagaagtattgggccgagcgatcatcgttaagaagctcaacatgctgccctttgagtgcgttgcccgcggttacctcaccggttccggcttgaaggaatacaacgctaacggcaccgtgtgcggcatcgagctgccagaaggcttggttgaggcgtcgcgtctgccagagccaattttcaccccagccaccaaggcagagcagggcgaccacgatgaaaacgtcagcttcgagcgcgtggtgcaggaccttggccaagagcgcgcagagcagcttcgcgatgaaaccctgcgcatctactccgccgccgccaagattgccgaagaaaagggcatcatcttggctgatacgaagtttgaattcggccttgattccgaaggcaatctggtcttgggcgatgaagtacttacgcctgattcctcccggtactggccagcagacacctacgcggaaggcattgtgcagcccagctttgacaagcagtacgtgcgcaactggttgacctcggaggaatccggctgggatgtggagtcggaaacccagccgccagtgcttcccgatgacatcgtcgccgccacccgcctgcgctacatcgaggcttatgagcgcttgtccggcaagcgtttcatcgacttcattggcggttaa

SEQ ID NO: 35 - DNA, 888 bp, synthetic construct
  source 1..888: mol_type = other DNA
atgcgcccacagctttctgattatcagcacgtatcctccggcaaagtccgcgatatctacgaagtagatgacaacactttgctcatggtggtcaccgaccgcatctccgcctatgacttcgcactagagccagccatccccgataaaggccgggttcttaccgcaaccaccatgttcttcttcgacgccatcgatttcccgaacccattggcaggacccatcgatgatgcgcggattccagaagaagtattgggccgagcgatcatcgttaagaagctcaacatgctgccctttgagtgcgttgcccgcggttacctcaccggttccggcttgaaggaatacaacgctaacggcaccgtgtgcggcatcgagctgccagaaggcttggttgaggcgtcgcgtctgccagagccaattttcaccccagccaccaaggcagagcagggcgaccacgatgaaaacgtcagcttcgagcgcgtggtgcaggaccttggccaagagcgcgcagagcagcttcgcgatgaaaccctgcgcatctactccgccgccgccaagattgccgaagaaaagggcatcatcttggctgatacgaagtttgaattcggccttgattccgaaggcaatctggtcttgggcgatgaagtacttacgcctgattcctcccggtactggccagcagacacctacgcggaaggcattgtgcagcccagctttgacaagcagtacgtgcgcaactggttgacctcggaggaatccggctgggatgtggagtcggaaacccagccgccagtgcttcccgatgacatcgtcgccgccacccgcctgcgctacatcgaggcttatgagcgcttgtccggcaagcgtttcatcgacttcattggcggttaa

SEQ ID NO: 36 - DNA, 888 bp, synthetic construct
  source 1..888: mol_type = other DNA
atgcgcccacagctttctgattatcagcacgtatcctccggcaaagtccgcgatatctacgaagtagatgacaacactttgctcatggtggtcaccgaccgcatctccgcctatgacttcgcactagagccagccatccccgataaaggccgggttcttaccgcaaccaccatgttcttcttcgacgccatcgatttcccgaactcgttggcaggacccatcgatgatgcgcggattccagaagaagtattgggccgagcgatcatcgttaagaagctcaacatgctgccctttgagtgcgttgcccgcggttacctcaccggttccggcttgaaggaatacaacgctaacggcaccgtgtgcggcatcgagctgccagaaggcttggttgaggcgtcgcgtctgccagagccaattttcaccccagccaccaaggcagagcagggcgaccacgatgaaaacgtcagcttcgagcgcgtggtgcaggaccttggccaagagcgcgcagagcagcttcgcgatgaaaccctgcgcatctactccgccgccgccaagattgccgaagaaaagggcatcatcttggctgatacgaagtttgaattcggccttgattccgaaggcaatctggtcttgggcgatgaagtacttacgcctgattcctcccggtactggccagcagacacctacgcggaaggcattgtgcagcccagctttgacaagcagtacgtgcgcaactggttgacctcggaggaatccggctgggatgtggagtcggaaacccagccgccagtgcttcccgatgacatcgtcgccgccacccgcctgcgctacatcgaggcttatgagcgcttgtccggcaagcgtttcatcgacttcattggcggttaa

SEQ ID NO: 37 - DNA, 5802 bp, synthetic construct
  source 1..5802: mol_type = other DNA
gttcgcttgctgtccataaaaccgcccagtctagctatcgccatgtaagcccactgcaagctacctgctttctctttgcgcttgcgttttcccttgtccagatagcccagtagctgacattcatccggggtcagcaccgtttctgcggactggctttctacgtgttccgcttcctttagcagcccttgcgccctgagtgcttgcggcagcgtgaagctagcttttatcgccattcgccattcaggctgcgcaactgttgggaagggcgatcggtgcgggcctcttcgctattacgccagctggcgaaagggggatgtgctgcaaggcgattaagttgggtaacgccagggttttcccagtcacgacgttgtaaaacgacggccagtgaattcgagctcggtacccggggatcctctagagtcgacctgcaggcatgcaagcttggcgtaatcatggtcatagctgtttcctgtgtgaaattgttatccgctcacaattccacacaacatacgagccggaagcataaagtgtaaagcctggggtgcctaatgagtgagctaactcacattaattgcgttgcgctcactgcccgctttccagtcgggaaacctgtcgtgccagctgcattaatgaatcggccaacgcgcggggagaggcggtttgcgtattgggcgctcttccgcttcctcgctcactgactcgctgcgctcggtcgttcggctgcggcgagcggtatcagctcactcaaaggcggtaatacggttatccacagaatcaggggataacgcaggaaagaacatgtgagcaaaaggccagcaaaaggccaggaaccgtaaaaaggccgcgttgctggcgtttttccataggctccgcccccctgacgagcatcacaaaaatcgacgctcaagtcagaggtggcgaaacccgacaggactataaagataccaggcgtttccccctggaagctccctcgtgcgctctcctgttccgaccctgccgcttaccggatacctgtccgcctttctcccttcgggaagcgtggcgctttctcaatgctcacgctgtaggtatctcagttcggtgtaggtcgttcgctccaagctgggctgtgtgcacgaaccccccgttcagcccgaccgctgcgccttatccggtaactatcgtcttgagtccaacccggtaagacacgacttatcgccactggcagcagccactggtaacaggattagcagagcgaggtatgtaggcggtgctacagagttcttgaagtggtggcctaactacggctacactagaaggacagtatttggtatctgcgctctgctgaagccagttaccttcggaaaaagagttggtagctcttgatccggcaaacaaaccaccgctggtagcggtggtttttttgtttgcaagcagcagattacgcgcagaaaaaaaggatctcaagaagatcctttgatcttttctacggggtctgacgctcagtggaacgaaaactcacgttaagggattttggtcatgagattatcaaaaaggatcttcacctagatccttttggggtgggcgaagaactccagcatgagatccccgcgctggaggatcatccagccctgatagaaacagaagccactggagcacctcaaaaacaccatcatacactaaatcagtaagttggcagcatcacccgacgcactttgcgccgaataaatacctgtgacggaagatcacttcgcagaataaataaatcctggtgtccctgttgataccgggaagccctgggccaacttttggcgaaaatgagacgttgatcggcacgtaagaggttccaactttcaccataatgaaataagatcactaccgggcgtattttttgagttatcgagattttcaggagctgatagaaacagaagccactggagcacctcaaaaacaccatcatacactaaatcagtaagttggcagcatcacccgacgcactttgcgccgaataaatacctgtgacggaagatcacttcgcagaataaataaatcctggtgtccctgttgataccgggaagccctgggccaacttttggcgaaaatgagacgttgatcggcacgtaagaggttccaactttcaccataatgaaataagatcactaccgggcgtattttttgagttatcgagattttcaggagctctttggcatcgtctctcgcctgtcccctcagttcagtaatttcctgcatttgcctgtttccagtcggtagatattccacaaaacagcagggaagcagcgcttttccgctgcataaccctgcttcggggtcattatagcgattttttcggtatatccatcctttttcgcacgatatacaggattttgccaaagggttcgtgtagactttccttggtgtatccaacggcgtcagccgggcaggataggtgaagtaggcccacccgcgagcgggtgttccttcttcactgtcccttattcgcacctggcggtgctcaacgggaatcctgctctgcgaggctggccggctaccgccggcgtaacagatgagggcaagcggatggctgatgaaaccaagccaaccaggaagggcagcccacctatcaaggtgtactgccttccagacgaacgaagagcgattgaggaaaaggcggcggcggccggcatgagcctgtcggcctacctgctggccgtcggccagggctacaaaatcacgggcgtcgtggactatgagcacgtccgcgagggcgtcccggaaaacgattccgaagcccaacctttcatagaaggcggcggtggaatcgaaatctcgtgatggcaggttgggcgtcgcttggtcggtcatttcgaaaaaggttaggaatacggttagccatttgcctgcttttatatagttcatatgggattcacctttatgttgataagaaataaaagaaaatgccaataggatatcggcattttcttttgcgtttttatttgttaactgttaattgtccttgttcaaggatgctgtctttgacaacagatgttttcttgcctttgatgttcagcaggaagctcggcgcaaacgttgattgtttgtctgcgtagaatcctctgtttgtcatatagcttgtaatcacgacattgtttcctttcgcttgaggtacagcgaagtgtgagtaagtaaaggttacatcgttaggcggatcaagatccatttttaacacaaggccagttttgttcagcggcttgtatgggccagttaaagaattagaaacataaccaagcatgtaaatatcgttagacgtaatgccgtcaatcgtcatttttgatccgcgggagtcagtgaacaggtaccatttgccgttcattttaaagacgttcgcgcgttcaatttcatctgttactgtgttagatgcaatcagcggtttcatcacttttttcagtgtgtaatcatcgtttagctcaatcataccgagagcgccgtttgctaactcagccgtgcgttttttatcgctttgcagaagtttttgactttcttgacggaagaatgatgtgcttttgccatagtatgctttgttaaataaagattcttcgccttggtagccatcttcagttccagtgtttgcttcaaatactaagtatttgtggcctttatcttctacgtagtgaggatctctcagcgtatggttgtcgcctgagctgtagttgccttcatcgatgaactgctgtacattttgatacgtttttccgtcaccgtcaaagattgatttataatcctctacaccgttgatgttcaaagagctgtctgatgctgatacgttaacttgtgcagttgtcagtgtttgtttgccgtaatgtttaccggagaaatcagtgtagaataaacggatttttccgtcagatgtaaatgtggctgaacctgaccattcttgtgtttggtcttttaggatagaatcatttgcatcgaatttgtcgctgtctttaaagacgcggccagcgtttttccagctgtcaatagaagtttcgccgactttttgatagaacatgtaaatcgatgtgtcatccgcatttttaggatctccggctaatgcaaagacgatgtggtagccgtgatagtttgcgacagtgccgtcagcgttttgtaatggccagctgtcccaaacgtccaggccttttgcagaagagatatttttaattgtggacgaatcaaattcagaaacttgatatttttcatttttttgctgttcagggatttgcagcatatcatggcgtgtaatatgggaaatgccgtatgtttccttatatggcttttggttcgtttctttcgcaaacgcttgagttgcgcctcctgccagcagtgcggtagtaaaggttaatactgttgcttgttttgcaaactttttgatgttcatcgttcatgtctccttttttatgtactgtgttagcggtctgcttcttccagccctcctgtttgaagatggcaagttagttacgcacaataaaaaaagacctaaaatatgtaaggggtgacgccaaagtatacactttgccctttacacattttaggtcttgcctgctttatcagtaacaaacccgcgcgatttacttttcgacctcattctattagactctcgtttggattgcaactggtctattttcctcttttgtttgatagaaaatcataaaaggatttgcagactacgggcctaaagaactaaaaaatctatctgtttcttttcattctctgtattttttatagtttctgttgcatgggcataaagttgcctttttaatcacaattcagaaaatatcataatatctcatttcactaaataatagtgaacggcaggtatatgtgatgggttaaaaaggatcaccccagagtcccgctcagaagaactcgtcaagaaggcgatagaaggcgatgcgctgcgaatcgggagcggcgataccgtaaagcacgaggaagcggtcagcccattcgccgccaagctcttcagcaatatcacgggtagccaacgctatgtcctgatagcggtccgccacacccagccggccacagtcgatgaatccagaaaagcggccattttccaccatgatattcggcaagcaggcatcgccatgggtcacgacgagatcctcgccgtcgggcatccgcgccttgagcctggcgaacagttcggctggcgcgagcccctgatgctcttcgtccagatcatcctgatcgacaagaccggcttccatccgagtacgtgctcgctcgatgcgatgtttcgcttggtggtcgaatgggcaggtagccggatcaagcgtatgcagccgccgcattgcatcagccatgatggatactttctcggcaggagcaaggtgagatgacaggagatcctgccccggcacttcgcccaatagcagccagtcccttcccgcttcagtgacaacgtcgagacagctgcgcaaggaacgcccgtcgtggccagccacgatagccgcgctgcctcgtcttggagttcattcagggcaccggacaggtcggtcttgacaaaaagaaccgggcgcccctgcgctgacagccggaacacggcggcatcagagcagccgattgtctgttgtgcccagtcatagccgaatagcctctccacccaagcggccggagaacctgcgtgcaatccatcttgttcaatcatgcgaaacgatcctcatcctgtctcttgatcagatcttgatcccctgcgccatcagatccttggcggcaagaaagccatccagtttactttgcagggcttcccaaccttaccagagggcgccccagctggcaattccg